European Patent Specification EP 3 953 375 B9, published October 4, 2023. Title: NOVEL PSMA SPECIFIC BINDING PROTEINS FOR CANCER DIAGNOSIS AND TREATMENT. Applicant: Navigo Proteins GmbH. The sequence listing filed with the application follows.

SEQUENCE LISTING (78 sequences)

SEQ ID NO: 1 - protein, 76 aa, Artificial Sequence
  ubiquitin wildtype
MQIFVKTLTGKTITLEVEPSDTIENVKAKIQDKEGIPPDQQRLIWAGKQLEDGRTLSDYNIQKESTLHLVLRLRAA

SEQ ID NO: 2 - protein, 152 aa, Artificial Sequence
  bis-ubiquitin
MQIFVKTLTGKTITLEVEPSDTIENVKAKIQDKEGIPPDQQRLIWAGKQLEDGRTLSDYNIQKESTLHLVLRLRAAMQIFVKTLTGKTITLEVEPSDTIENVKAKIQDKEGIPPDQQRLIWAGKQLEDGRTLSDYNIQKESTLHLVLRLRAA

SEQ ID NO: 3 - protein, 152 aa, Artificial Sequence
  Affilin 162462 (CID167521)
MQIFVRTPTGKTITLEVEPSDTIENVKAKIQDKEGIPPDQQRLIWAGKQLEDGRTLSDYNIGFAHRLHLVLRLRAAMQIFVMTQTGKTITLEVEPSDTIENVKAKIQDKEGIPPDQQRLIWAGKQLEDGRTLSDYNIWTTTFLHLVLRLRAA

SEQ ID NO: 4 - protein, 152 aa, Artificial Sequence
  Affilin 191871
MQIFVRTQTGKTITLEVEPSDTIENVKAKIQDKEGIPPDQQRLIWAGKQLEDGRTLSDYNIGWAHRLHLVLRLRAAMQIFVHTNTGKTITLEVEPSDTIENVKAKIQDKEGIPPDQQRLIWAGKQLEDGRTLSDYNIWTETILHLVLRLRAA

SEQ ID NO: 5 - protein, 155 aa, Artificial Sequence
  Affilin 191871 with c-terminal coupling site
MQIFVRTQTGKTITLEVEPSDTIENVKAKIQDKEGIPPDQQRLIWAGKQLEDGRTLSDYNIGWAHRLHLVLRLRAAMQIFVHTNTGKTITLEVEPSDTIENVKAKIQDKEGIPPDQQRLIWAGKQLEDGRTLSDYNIWTETILHLVLRLRAASAC

SEQ ID NO: 6 - protein, 152 aa, Artificial Sequence
  Affilin 161421
MQIFVRTDTGKTITLEVEPSDTIENVKAKIQDKEGIPPDQQRLIWAGKQLEDGRTLSDYNIGWAHRLHLVLRLRAAMQIFVMTQTGKTITLEVEPSDTIENVKAKIQDKEGIPPDQQRLIWAGKQLEDGRTLSDYNIWTTTFLHLVLRLRAA

SEQ ID NO: 7 - protein, 152 aa, Artificial Sequence
  Affilin 164052
MQIFVRTGTGKTITLEVEPSDTIENVKAKIQDKEGIPPDQQRLIWAGKQLEDGRTLSDYNIGFAHRLHLVLRLRAAMQIFVMTQTGKTITLEVEPSDTIENVKAKIQDKEGIPPDQQRLIWAGKQLEDGRTLSDYNIWTTTFLHLVLRLRAA

SEQ ID NO: 8 - protein, 152 aa, Artificial Sequence
  Affilin 161438
MQIFVRTHTGKTITLEVEPSDTIENVKAKIQDKEGIPPDQQRLIWAGKQLEDGRTLSDYNISFAHRLHLVLRLRAAMQIFVMTRTGKTITLEVEPSDTIENVKAKIQDKEGIPPDQQRLIWAGKQLEDGRTLSDYNIWTTTFLHLVLRLRAA

SEQ ID NO: 9 - protein, 152 aa, Artificial Sequence
  Affilin 164058
MQIFVRTITGKTITLEVEPSDTIENVKAKIQDKEGIPPDQQRLIWAGKQLEDGRTLSDYNIGFAHRLHLVLRLRAAMQIFVMTQTGKTITLEVEPSDTIENVKAKIQDKEGIPPDQQRLIWAGKQLEDGRTLSDYNIWTTTFLHLVLRLRAA

SEQ ID NO: 10 - protein, 152 aa, Artificial Sequence
  Affilin 185036
MQIFVRTLTGKTITLEVEPSDTIENVKAKIQDKEGIPPDQQRLIWAGKQLEDGRTLSDYNIGFAHRLHLVLRLRAAMQIFVLTQTGKTITLEVEPSDTIENVKAKIQDKEGIPPDQQRLIWAGKQLEDGRTLSDYNIWTPSILHLVLRLRAA

SEQ ID NO: 11 - protein, 152 aa, Artificial Sequence
  Affilin 192444
MQIFVRTLTGKTITLEVEPSDTIENVKAKIQDTEGIPPDQQRLIWAGKQLEDGRTLSDYNIGFAHRLHLVLRLRAAMQIFVLTQTGKTITLEVEPSDTIENVKAKIQDKEGIPPDQQRLIWAGTQLEDGRTLSDYNIWTPSILHLVLRLRAA

SEQ ID NO: 12 - protein, 152 aa, Artificial Sequence
  Affilin 191822
MQIFVRTLTGQTITLEVEPSDTIENVKAKIQDKEGIPPDQQRLIWAGKQLADGRTLSDYNIGFAHRLHLVLRLRAAMQIFVLTQTGKTITLEVEPSDTIENVKAKIQDKEGIPPDQQRLIWAGKQLEDGRTLSDYNIWTPSILHLVLRLRAA

SEQ ID NO: 13 - protein, 152 aa, Artificial Sequence
  Affilin 185678
MQIFVRTLTGKTITLEVEPSDTIENVKAKIQDKEGIPPDQQRLIWAGKQLEDGRTLSDYNIGFAHRLHLVLRLRAAMQIFVMTQTGKTITLEVEPSDTIENVKAKIQDKEGIPPDQQRLIWAGKQLEDGRTLSDYNIGHEYLLHLVLRLRAA

SEQ ID NO: 14 - protein, 152 aa, Artificial Sequence
  Affilin 185152
MQIFVRTMTGKTITLEVEPSDTIENVKAKIQDKEGIPPDQQRLIWAGKQLEDGRTLSDYNIGFAHRLHLVLRLRAAMQIFVMTQTGKTITLEVEPSDTIENVKAKIQDKEGIPPDQQRLIWAGKQLEDGRTLSDYNIGDGDVLHLVLRLRAA

SEQ ID NO: 15 - protein, 152 aa, Artificial Sequence
  Affilin 164668  (164000)
MQIFVRTMTGKTITLEVEPSDTIENVKAKIQDKEGIPPDQQRLIWAGKQLEDGRTLSDYNIGFAHRLHLVLRLRAAMQIFVMTQTGKTITLEVEPSDTIENVKAKIQDKEGIPPDQQRLIWAGKQLEDGRTLSDYNIWTTTFLHLVLRLRAA

SEQ ID NO: 16 - protein, 152 aa, Artificial Sequence
  Affilin 185071
MQIFVRTMTGKTITLEVEPSDTIENVKAKIQDKEGIPPDQQRLIWAGKQLEDGRTLSDYNIWGGHRLHLVLRLRAAMQIFVLTQTGKTITLEVEPSDTIENVKAKIQDKEGIPPDQQRLIWAGKQLEDGRTLSDYNIWTPSILHLVLRLRAA

SEQ ID NO: 17 - protein, 152 aa, Artificial Sequence
  Affilin 157424
MQIFVRTPTGKTITLEVEPSDTIENVKAKIQDKEGIPPDQQRLIWAGKQLEDGRTLSDYNIQPAHQLHLVLRLCAAMQIFVMTQTGKTITLEVEPSDTIENVKAKIQDKEGIPPDQQRLIWAGKQLEDGRTLSDYNIWTTTFLHLVLRLRAA

SEQ ID NO: 18 - protein, 152 aa, Artificial Sequence
  Affilin 157423
MQIFVRTPTGKTITLEVEPSDTIENVKAKIQDKEGIPPDQQRLIWAGKQLEDGRTLSDYNIQPAHQLHLVLRLRAAMQIFVMTRTGKTITLEVEPSDTIENVKAKIQDKEGIPPDQQRLIWAGKQLEDGRTLSDYNIWTTTFLHLVLRLRAA

SEQ ID NO: 19 - protein, 152 aa, Artificial Sequence
  Affilin 161644
MQIFVRTPTGKTITLEVEPSDTIENVKAKIQDKEGIPPDQQRLIWAGKQLEDGRTLSDYNISYAHRLHLVLRLRAAMQIFVMTQTGKTITLEVEPSDTIENVKAKIQDKEGIPPDQQRLIWAGKQLEDGRTLSDYNIWTTTFLHLVLRLRAA

SEQ ID NO: 20 - protein, 152 aa, Artificial Sequence
  Affilin 191829
MQIFVRTQTGKTITLEVEPSDTIENVKAKIQDKEGIPPDQQRLIWAGKQLEDGRTLSDYNIGWAHRLHLVLRLRAAMQIFVATFTGKTITLEVEPSDTIENVKAKIQDKEGIPPDQQRLIWAGKQLEDGRTLSDYNIWTPTILHLVLRLRAA

SEQ ID NO: 21 - protein, 152 aa, Artificial Sequence
  Affilin 185113
MQIFVRTWTGKTITLEVEPSDTIENVKAKIQDKEGIPPDQQRLIWAGKQLEDGRTLSDYNIGFAHRLHLVLRLRAAMQIFVMTHTGKTITLEVEPSDTIENVKAKIQDKEGIPPDQQRLIWAGKQLEDGRTLSDYNIGDGDVLHLVLRLRAA

SEQ ID NO: 22 - protein, 152 aa, Artificial Sequence
  Affilin 185104
MQIFVRTWTGKTITLEVEPSDTIENVKAKIQDKEGIPPDQQRLIWAGKQLEDGRTLSDYNIGFAHRLHLVLRLRAAMQIFVMTQTGKTITLEVEPSDTIENVKAKIQDKEGIPPDQQRLIWAGKQLEDGRTLSDYNIGDGDVLHLVLRLRAA

SEQ ID NO: 23 - protein, 152 aa, Artificial Sequence
  Affilin 162633
MQIFVRTWTGKTITLEVEPSDTIENVKAKIQDKEGIPPDQQRLIWAGKQLEDGRTLSDYNIWWADRLHLVLRLRAAMQIFVMTQTGKTITLEVEPSDTIENVKAKIQDKEGIPPDQQRLIWAGKQLEDGRTLSDYNIWTTTFLHLVLRLRAA

SEQ ID NO: 24 - protein, 152 aa, Artificial Sequence
  Affilin 163970
MQIFVWTPTGKTITLEVEPSDTIENVKAKIQDKEGIPPDQQRLIWAGKQLEDGRTLSDYNIGFAHLLHLVLRLRAAMQIFVMTQTGKTITLEVEPSDTIENVKAKIQDKEGIPPDQQRLIWAGKQLEDGRTLSDYNIWTTTFLHLVLRLRAA

SEQ ID NO: 25 - protein, 82 aa, Artificial Sequence
  Affilin 164667 (161984)
MQIFVKTLTFEHPSFGKTITLEVEPSDTIENVKAKIQDKEGIPPDQQHLYWAGKQLEDGRTLSDYNIKHNTWLELMLFLRAA

SEQ ID NO: 26 - protein, 82 aa, Artificial Sequence
  Affilin 157434
MQIFVKTLTDMYRFMGKTITLEVEPSDTIENVKAKIQDKEGIPPDQQILWWAGKQLEDGRTLSDYNIVAYRPLYLTLALRAA

SEQ ID NO: 27 - protein, 82 aa, Artificial Sequence
  Afffilin 161717
MQIFVKTLTFEHHSFGKTITLEVEPSDTIENVKAKIQDKEGIPPDQQHLYWAGKQLEDGRTLSDYNIKHNTWLELMLFLRAA

SEQ ID NO: 28 - protein, 82 aa, Artificial Sequence
  Affilin 161776
MQIFVKTLTFEHKSFGKTITLEVEPSDTIENVKAKIQDKEGIPPDQQHLYWAGKQLEDGRTLSDYNIKHNTWLELMLFLRAA

SEQ ID NO: 29 - protein, 82 aa, Artificial Sequence
  Affilin 162055
MQIFVKTLTFEHNSFGKTITLEVEPSDTIENVKAKIQDKEGIPPDQQHLYWVGKQLEDGRTLSDYNIKHNTWLELMLFLRAA

SEQ ID NO: 30 - protein, 82 aa, Artificial Sequence
  Affilin 162102
MQIFVKTLTPIPPDWGKTITLEVEPSDTIENVKAKIQDKEGIPPDQQHLYWAGKQLEDGRTLSDYNIKHNTWLELMLFLRAA

SEQ ID NO: 31 - protein, 82 aa, Artificial Sequence
  Affilin 161912
MQIFVKTLTPPFAFWGKTITLEVEPSDTIENVKAKIQDKEGIPPDQQHLYWAGKQLEDGRTLSDYNIKHNTWLELMLFLRAA

SEQ ID NO: 32 - protein, 82 aa, Artificial Sequence
  Affilin 162034
MQIFVKTLTPQPPEFGKTITLEVEPSDTIENVKAKIQDKEGIPPDQQHLYWAGKQLEDGRTLSDYNIKHNTWLELMLFLRAA

SEQ ID NO: 33 - protein, 82 aa, Artificial Sequence
  Affilin 161843
MQIFVKTLTPQPPEWGKTITLEVEPSDTIENVKAKIQDKEGIPPDQQHLYWAGKQLEDGRTLSDYNIKHNTWLELMLFLRAA

SEQ ID NO: 34 - protein, 82 aa, Artificial Sequence
  Affilin 161374
MQIFVKTLTPQPPEYGKTITLEVEPSDTIENVKAKIQDKEGIPPDQQHLYWAGKQLEDGRTLSDYNIKHNTWLELMLFLRAA

SEQ ID NO: 35 - protein, 76 aa, Artificial Sequence
  Affilin 187093
MQIFVWTREFKQITLEVEPSDTIENVKAKIQDKEGIPPDQQMLFWKGKQLEDGRTLSDYNIWWNPNLSLNLDLRAA

SEQ ID NO: 36 - protein, 76 aa, Artificial Sequence
  Affilin 187092
MQIFVYTAELKQITLEVEPSDTIENVKAKIQDKEGIPPDQQMLFWKGKQLEDGRTLSDYNIWWNPNLSLNLDLRAA

SEQ ID NO: 37 - protein, 76 aa, Artificial Sequence
  Affilin 187064
MQIFVYTKQLKQITLEVEPSDTIENVKAKIQDKEGIPPDQQMLFWKGKQLEDGRTLSDYNIWWNPNLSLNLDLRAA

SEQ ID NO: 38 - protein, 76 aa, Artificial Sequence
  Affilin 187154
MQIFVYTRALKQITLEVGPSDTIENVKAKIRDKEGIPPDQQMLFWKGKQLEDGRTLSDYNIWWNPNLSLDLDLRAA

SEQ ID NO: 39 - protein, 76 aa, Artificial Sequence
  Affilin 187165
MQIFVYTRALKQITLEVEPSDTVENVKAKIQDKEGIPPDQQMLFWKGKQLEDGRTLSDYNIWWNPNLSLDLDLRAA

SEQ ID NO: 40 - protein, 76 aa, Artificial Sequence
  Affilin 187191
MQIFVYTRALKQITLEVEPSDTIENVKAKIQDKEGIPPDQQMLFWKGRQLEDGRTLSDYNIWWNPNLSLNLDLRAA

SEQ ID NO: 41 - protein, 76 aa, Artificial Sequence
  Affilin 187210
MQIFVYTRALKQITLEVEPSDTIENVKAKIQDREGIPPDQQMLFWKGKQLEDGRTLSDYNIWWNPNLSLNLDLRAA

SEQ ID NO: 42 - protein, 76 aa, Artificial Sequence
  Affilin 187131
MQIFVYTRALKQITLEVEPSDTIENVKAKIQDKEGIPPDQQMLFWKGKQLEDGRTLSDYNIWWNPNLSLNLGLRAA

SEQ ID NO: 43 - protein, 76 aa, Artificial Sequence
  Affilin 187170
MQIFVYTRALKQITLEVEPSDTIENVKAKIQDKEGIPPDQQMLFWKGKQLEDGRTLSDYNIWWNPNLSLNLNLRAA

SEQ ID NO: 44 - protein, 76 aa, Artificial Sequence
  Affilin 187096
MQIFVYTRELKQITLEVEPSDTIENVKAKIQDKEGIPPDQQMLFWKGKQLEDGRTLSDYNIWWNPNLSLNLDLRAA

SEQ ID NO: 45 - protein, 76 aa, Artificial Sequence
  Affilin 181514
MQIFVYTRVLKQITLEVEPSDTIENVKAKIQDKEGIPPDQQKLKWKGKQLEDGRTLSDYNIWWNPNLSLNLDLRAA

SEQ ID NO: 46 - protein, 76 aa, Artificial Sequence
  Affilin 181515
MQIFVYTRVLKQITLEVEPSDTIENVKAKIQDKEGIPPDQQMLFWKGKQLEDGRTLSDYNIWWNPNLSLNLDLRAA

SEQ ID NO: 47 - protein, 76 aa, Artificial Sequence
  Affilin 187134
MQIFVYTRVLKQITLAVEPSDTIENVKAKIQDKEGIPPDQQMLFWKGKQLEDGRTLSDYNIWWNPNLSLNLDLRAA

SEQ ID NO: 48 - protein, 76 aa, Artificial Sequence
  Affilin 187186
MQIFVYTRVLKQITLEVEPSDTIENVKARIQDKEGIPPDQQMLFWKGKQLEDGRTLSDYNIWWNPNLSLNLDLRAA

SEQ ID NO: 49 - protein, 76 aa, Artificial Sequence
  Affilin 187283
MQIFVYTRVLKQITLEVEPSDTIENVKAKIQDKEGIPPDQQMLFWKGKQLEDGRTLSDYNIWWNPNLSLNRDLRAA

SEQ ID NO: 50 - protein, 76 aa, Artificial Sequence
  Affilin 187295
MQIFVYTRVLKQITLEVEPSDTIENVKAKIQDKEGIPPDQQMLFWKGKQLEDGRTLSDYNIWWNPNLSLNLDRRAA

SEQ ID NO: 51 - protein, 76 aa, Artificial Sequence
  Affilin 187178
MQIFVYTRVLKQITLEVEPSDTIENVKAKIQDKEGTPPDQQTLFWRGKQLEDGRTLSDYNIWWNPNLSLNLDLRAA

SEQ ID NO: 52 - protein, 404 aa, Artificial Sequence
  homodimer of 167528 (162462)
MQIFVRTPTGKTITLEVEPSDTIENVKAKIQDKEGIPPDQQRLIWAGKQLEDGRTLSDYNIGFAHRLHLVLRLRAAMQIFVMTQTGKTITLEVEPSDTIENVKAKIQDKEGIPPDQQRLIWAGKQLEDGRTLSDYNIWTTTFLHLVLRLRAASAPAASPSPAAPAPSPASPAPASPASAPSAPASAPPAASAMQIFVRTPTGKTITLEVEPSDTIENVKAKIQDKEGIPPDQQRLIWAGKQLEDGRTLSDYNIGFAHRLHLVLRLRAAMQIFVMTQTGKTITLEVEPSDTIENVKAKIQDKEGIPPDQQRLIWAGKQLEDGRTLSDYNIWTTTFLHLVLRLRAASAPAPSAPAASAPPAPAAPCAPAAPASAPAPASAPAASPCPAAPAPSPASPAPASPASAP

SEQ ID NO: 53 - protein, 264 aa, Artificial Sequence
  homomer 161984 (164661)
MQIFVKTLTFEHPSFGKTITLEVEPSDTIENVKAKIQDKEGIPPDQQHLYWAGKQLEDGRTLSDYNIKHNTWLELMLFLRAASAPAASPSPAAPAPSPASPAPASPASAPSAPASAPPAASAMQIFVKTLTFEHPSFGKTITLEVEPSDTIENVKAKIQDKEGIPPDQQHLYWAGKQLEDGRTLSDYNIKHNTWLELMLFLRAASAPAPSAPAASAPPAPAAPCAPAAPASAPAPASAPAASPCPAAPAPSPASPAPASPASAP

SEQ ID NO: 54 - protein, 334 aa, Artificial Sequence
  heterodimer 42 of 161984 und 162462 (CID167526)
MQIFVKTLTFEHPSFGKTITLEVEPSDTIENVKAKIQDKEGIPPDQQHLYWAGKQLEDGRTLSDYNIKHNTWLELMLFLRAASAPAASPSPAAPAPSPASPAPASPASAPSAPASAPPAASAMQIFVRTPTGKTITLEVEPSDTIENVKAKIQDKEGIPPDQQRLIWAGKQLEDGRTLSDYNIGFAHRLHLVLRLRAAMQIFVMTQTGKTITLEVEPSDTIENVKAKIQDKEGIPPDQQRLIWAGKQLEDGRTLSDYNIWTTTFLHLVLRLRAASAPAPSAPAASAPPAPAAPCAPAAPASAPAPASAPAASPCPAAPAPSPASPAPASPASAP

SEQ ID NO: 55 - protein, 334 aa, Artificial Sequence
  heterodimer 24 162462 und 161984 (CID167525)
MQIFVRTPTGKTITLEVEPSDTIENVKAKIQDKEGIPPDQQRLIWAGKQLEDGRTLSDYNIGFAHRLHLVLRLRAAMQIFVMTQTGKTITLEVEPSDTIENVKAKIQDKEGIPPDQQRLIWAGKQLEDGRTLSDYNIWTTTFLHLVLRLRAASAPAASPSPAAPAPSPASPAPASPASAPSAPASAPPAASAMQIFVKTLTFEHPSFGKTITLEVEPSDTIENVKAKIQDKEGIPPDQQHLYWAGKQLEDGRTLSDYNIKHNTWLELMLFLRAASAPAPSAPAASAPPAPAAPCAPAAPASAPAPASAPAASPCPAAPAPSPASPAPASPASAP

SEQ ID NO: 56 - protein, 5 aa, Artificial Sequence
  motif
GFAHR

SEQ ID NO: 57 - protein, 5 aa, Artificial Sequence
  motif
GWAHR

SEQ ID NO: 58 - protein, 5 aa, Artificial Sequence
  motif
WTTTF

SEQ ID NO: 59 - protein, 5 aa, Artificial Sequence
  motif
KHNTW

SEQ ID NO: 60 - protein, 5 aa, Artificial Sequence
  motif
VAYRP

SEQ ID NO: 61 - protein, 5 aa, Artificial Sequence
  motfi
WWNPN

SEQ ID NO: 62 - protein, 40 aa, Artificial Sequence
  linker
SAPAASPSPAAPAPSPASPAPASPASAPSAPASAPPAASA

SEQ ID NO: 63 - protein, 21 aa, Artificial Sequence
  linker
PAAPAPSPASPAPASPASAPS

SEQ ID NO: 64 - protein, 61 aa, Artificial Sequence
  coupling domain
SAPAPSAPAASAPPAPAAPCAPAAPASAPAPASAPAASPCPAAPAPSPASPAPASPASAPS

SEQ ID NO: 65 - protein, 40 aa, Artificial Sequence
  coupling domain
SAPAPSAPAASAPPAPAAPCAPAAPASAPAPASAPAASPC

SEQ ID NO: 66 - protein, 20 aa, Artificial Sequence
  coupling domain
SAPAPSAPAASAPPAPAAPC

SEQ ID NO: 67 - protein, 20 aa, Artificial Sequence
  coupling domain
APAAPASAPAPASAPAASPC

SEQ ID NO: 68 - protein, 33 aa, Artificial Sequence
  coupling domain
SAPAPSAPAASAPPAPAAPAAPAAPASAPAPAC

SEQ ID NO: 69 - protein, 33 aa, Artificial Sequence
  coupling domain
APAASPSPAAPAPSPASPAPASPASAPSAPASC

SEQ ID NO: 70 - protein, 98 aa, Artificial Sequence
  coupling domain
SAPAPSAPAASAPPAPAAPAAPAAPASAPAPAPAPAASPSPAAPAPSPAAPAPASPASAPSAPASAPPAAPSAAASPAPSAPAPAASPAAAPASAAPA

SEQ ID NO: 71 - protein, 10 aa, Artificial Sequence
  strep
SAWSHPQFEK

SEQ ID NO: 72 - protein, 5 aa, Artificial Sequence
  motif
SFAHR

SEQ ID NO: 73 - protein, 5 aa, Artificial Sequence
  motif
SYAHR

SEQ ID NO: 74 - protein, 5 aa, Artificial Sequence
  motif
GFAHL

SEQ ID NO: 75 - protein, 5 aa, Artificial Sequence
  motif
WTPSI

SEQ ID NO: 76 - protein, 5 aa, Artificial Sequence
  motif
WTETI

SEQ ID NO: 77 - protein, 5 aa, Artificial Sequence
  motif
GDGDV

SEQ ID NO: 78 - protein, 8 aa, Artificial Sequence
  FlagTag
DYKDDDDK